European Patent Application EP 4 290 228 A2, published December 13, 2023. Title: Compositions and Methods for Improving Nanopore Sequencing. Applicant: University of Washington through its Center for Commercialization. The sequence listing filed with the application follows.

SEQUENCE LISTING (4 sequences)

SEQ ID NO: 1 - DNA, 93 bp, synthetic construct
  misc_feature 1..93: note = Synthetic
  misc_feature 14: note = Wheren N at position 14 = X representing an abasic residue
  source 1..93: mol_type = other DNA
aaaaaaaccttccnagaccaatcaagcaactaattaagtaacgaatgaaggaacaaataaagaaaaccaagcattctcatgcaggtcgtagcc

SEQ ID NO: 2 - DNA, 43 bp, synthetic construct
  misc_feature 1..43: note = Synthetic
  misc_feature 37..43: note = Wherein N at positions 37-43 = X representing an abasic residue
  source 1..43: mol_type = other DNA
ttggttttctttatttgttccttcattcgttacttannnnnnn

SEQ ID NO: 3 - DNA, 55 bp, synthetic construct
  misc_feature 1..55: note = Synthetic
  source 1..55: mol_type = other DNA
gcgtacgcctacggttttccgtaggcgtacgcggctacgacctgcatgagaatgc

SEQ ID NO: 4 - DNA, 191 bp, synthetic construct
  misc_feature 1..191: note = Synthetic
  misc_feature 14: note = Wheren N at position 14 = X representing an abasic residue
  misc_feature 185..191: note = Wherein N at positions 185-191 = X representing an abasic residue
  source 1..191: mol_type = other DNA
aaaaaaaccttccnagaccaatcaagcaactaattaagtaacgaatgaaggaacaaataaagaaaaccaagcattctcatgcaggtcgtagccgcgtacgcctacggttttccgtaggcgtacgcggctacgacctgcatgagaatgcttggttttctttatttgttccttcattcgttacttannnnnnn